European Patent Specification EP 2 797 958 B1, published July 19, 2023. Title: Light Chain Bridged Bispecific Antibody. Applicant: Development Center for Biotechnology DCB-USA LLC. The sequence listing filed with the application follows.

SEQUENCE LISTING (4 sequences)

SEQ ID NO: 1 - protein, 105 aa, Homo sapiens [sequence omitted]

SEQ ID NO: 2 - protein, 106 aa, Homo sapiens
GQPKAAPSVTLFPPSSEELQANKATLVCLISDFYPGAVTVAWKADGSPVKAGVETTTPSKQSNNKYAASSYLSLTPEQWKSHRSYSCQVTHEGSTVEKTVAPTECS

SEQ ID NO: 3 - protein, 120 aa, Homo sapiens
VTHVFGSGTQLTVLSQPKATPSVTLFPPSSEELQANKATLVCLMNDFYPGILTVTWKADGTPITQGVEMTTPSKQSNNKYAASSYLSLTPEQWRSRRSYSCQVMHEGSTVEKTVAPTECS

SEQ ID NO: 4 - protein, 101 aa, Homo sapiens
TKGPSVFPLAPSSKSTSGGTAALGCLVKDYFPEPVTVSWNSGALTSGVHTFPAVLQSSGLYSLSSVVTVPSSSLGTQTYICNVNHKPSNTKVDKKAEPKSC